European Patent Application EP 4 574 170 A1, published June 25, 2025. Title: METHOD FOR TREATING A DISEASE OR DISORDER MEDIATED BY T-LYMPHOCYTES BEARING TRBV9 SEGMENT WITHIN T-CELL RECEPTOR. Applicant: JOINT STOCK COMPANY BIOCAD. Application WO PCT/RU2023/050196, filed August 18, 2023. The sequence listing filed with the application follows.

SEQUENCE LISTING (25 sequences)

SEQ ID NO: 1 - protein, 5 aa, synthetic construct
DYLVH

SEQ ID NO: 2 - protein, 17 aa, synthetic construct
WINTYTGTPTYADDFEG

SEQ ID NO: 3 - protein, 13 aa, synthetic construct
SWRRGLRGLGFDY

SEQ ID NO: 4 - protein, 13 aa, synthetic construct
SWRRGLRGIGFDY

SEQ ID NO: 5 - protein, 13 aa, synthetic construct
SWRRGIRGLGFDY

SEQ ID NO: 6 - protein, 13 aa, synthetic construct
SWRRGIRGIGFDY

SEQ ID NO: 7 - protein, 11 aa, synthetic construct
KASKSINKYLA

SEQ ID NO: 8 - protein, 7 aa, synthetic construct
DGSTLQS

SEQ ID NO: 9 - protein, 9 aa, synthetic construct
QQHNEYPPT

SEQ ID NO: 10 - protein, 122 aa, synthetic construct
QIQLVQSGPELREPGESVKLSCKASGYTFTDYLVHWVKQAPGKGLKWMGWINTYTGTPTYADDFEGRFVFSLEASASTANLQISNLKNEDTATYFCARSWRRGLRGLGFDYWGQGVFVTVSS

SEQ ID NO: 11 - protein, 122 aa, synthetic construct
QIQLVQSGPELREPGESVKLSCKASGYTFTDYLVHWVKQAPGKGLKWMGWINTYTGTPTYADDFEGRFVFSLEASASTANLQISNLKNEDTATYFCARSWRRGLRGIGFDYWGQGVFVTVSS

SEQ ID NO: 12 - protein, 122 aa, synthetic construct
QIQLVQSGPELREPGESVKLSCKASGYTFTDYLVHWVKQAPGKGLKWMGWINTYTGTPTYADDFEGRFVFSLEASASTANLQISNLKNEDTATYFCARSWRRGIRGLGFDYWGQGVFVTVSS

SEQ ID NO: 13 - protein, 122 aa, synthetic construct
QIQLVQSGPELREPGESVKLSCKASGYTFTDYLVHWVKQAPGKGLKWMGWINTYTGTPTYADDFEGRFVFSLEASASTANLQISNLKNEDTATYFCARSWRRGIRGIGFDYWGQGVFVTVSS

SEQ ID NO: 14 - protein, 122 aa, synthetic construct
QVQLVQSGSELKKPGESVKVSCKASGYTFTDYLVHWVRQAPGQGLEWMGWINTYTGTPTYADDFEGRFVFSLDTSVSTANLQISSLKAEDTAVYFCARSWRRGLRGIGFDYWGQGTLVTVSS

SEQ ID NO: 15 - protein, 122 aa, synthetic construct
QVQLVQSGPELKKPGESVKVSCKASGYTFTDYLVHWVRQAPGKGLEWMGWINTYTGTPTYADDFEGRFVFSLDTSASTANLQICSLKNEDTATYYCARSWRRGLRGIGFDYWGQGTLVTVSS

SEQ ID NO: 16 - protein, 107 aa, synthetic construct
DVQMTQSPYNLAASPGESVSINCKASKSINKYLAWYQQKPGKPNKLLIYDGSTLQSGIPSRFSGSGSGTDFTLTIRGLEPEDFGLYYCQQHNEYPPTFGAGTKLELK

SEQ ID NO: 17 - protein, 107 aa, synthetic construct
DIQMTQSPYSLSASVGDRVTITCKASKSINKYLAWFQQKPGKPNKLLIYDGSTLQSGVPSRFSGSGSGTDFTLTISSLEPEDFATYYCQQHNEYPPTFGQGTKLEIK

SEQ ID NO: 18 - protein, 452 aa, synthetic construct
QIQLVQSGPELREPGESVKLSCKASGYTFTDYLVHWVKQAPGKGLKWMGWINTYTGTPTYADDFEGRFVFSLEASASTANLQISNLKNEDTATYFCARSWRRGLRGLGFDYWGQGVFVTVSSASTKGPSVFPLAPSSKSTSGGTAALGCLVKDYFPEPVTVSWNSGALTSGVHTFPAVLQSSGLYSLSSVVTVPSSSLGTQTYICNVNHKPSNTKVDKKVEPKSCDKTHTCPPCPAPELLGGPSVFLFPPKPKDTLMISRTPEVTCVVVDVSHEDPEVKFNWYVDGVEVHNAKTKPREEQYNSTYRVVSVLTVLHQDWLNGKEYKCKVSNKALPAPIEKTISKAKGQPREPQVYTLPPSRDELTKNQVSLTCLVKGFYPSDIAVEWESNGQPENNYKTTPPVLDSDGSFFLYSKLTVDKSRWQQGNVFSCSVMHEALHNHYTQKSLSLSPGK

SEQ ID NO: 19 - protein, 452 aa, synthetic construct
QIQLVQSGPELREPGESVKLSCKASGYTFTDYLVHWVKQAPGKGLKWMGWINTYTGTPTYADDFEGRFVFSLEASASTANLQISNLKNEDTATYFCARSWRRGLRGIGFDYWGQGVFVTVSSASTKGPSVFPLAPSSKSTSGGTAALGCLVKDYFPEPVTVSWNSGALTSGVHTFPAVLQSSGLYSLSSVVTVPSSSLGTQTYICNVNHKPSNTKVDKKVEPKSCDKTHTCPPCPAPELLGGPSVFLFPPKPKDTLMISRTPEVTCVVVDVSHEDPEVKFNWYVDGVEVHNAKTKPREEQYNSTYRVVSVLTVLHQDWLNGKEYKCKVSNKALPAPIEKTISKAKGQPREPQVYTLPPSRDELTKNQVSLTCLVKGFYPSDIAVEWESNGQPENNYKTTPPVLDSDGSFFLYSKLTVDKSRWQQGNVFSCSVMHEALHNHYTQKSLSLSPGK

SEQ ID NO: 20 - protein, 452 aa, synthetic construct
QIQLVQSGPELREPGESVKLSCKASGYTFTDYLVHWVKQAPGKGLKWMGWINTYTGTPTYADDFEGRFVFSLEASASTANLQISNLKNEDTATYFCARSWRRGIRGLGFDYWGQGVFVTVSSASTKGPSVFPLAPSSKSTSGGTAALGCLVKDYFPEPVTVSWNSGALTSGVHTFPAVLQSSGLYSLSSVVTVPSSSLGTQTYICNVNHKPSNTKVDKKVEPKSCDKTHTCPPCPAPELLGGPSVFLFPPKPKDTLMISRTPEVTCVVVDVSHEDPEVKFNWYVDGVEVHNAKTKPREEQYNSTYRVVSVLTVLHQDWLNGKEYKCKVSNKALPAPIEKTISKAKGQPREPQVYTLPPSRDELTKNQVSLTCLVKGFYPSDIAVEWESNGQPENNYKTTPPVLDSDGSFFLYSKLTVDKSRWQQGNVFSCSVMHEALHNHYTQKSLSLSPGK

SEQ ID NO: 21 - protein, 452 aa, synthetic construct
QIQLVQSGPELREPGESVKLSCKASGYTFTDYLVHWVKQAPGKGLKWMGWINTYTGTPTYADDFEGRFVFSLEASASTANLQISNLKNEDTATYFCARSWRRGIRGIGFDYWGQGVFVTVSSASTKGPSVFPLAPSSKSTSGGTAALGCLVKDYFPEPVTVSWNSGALTSGVHTFPAVLQSSGLYSLSSVVTVPSSSLGTQTYICNVNHKPSNTKVDKKVEPKSCDKTHTCPPCPAPELLGGPSVFLFPPKPKDTLMISRTPEVTCVVVDVSHEDPEVKFNWYVDGVEVHNAKTKPREEQYNSTYRVVSVLTVLHQDWLNGKEYKCKVSNKALPAPIEKTISKAKGQPREPQVYTLPPSRDELTKNQVSLTCLVKGFYPSDIAVEWESNGQPENNYKTTPPVLDSDGSFFLYSKLTVDKSRWQQGNVFSCSVMHEALHNHYTQKSLSLSPGK

SEQ ID NO: 22 - protein, 452 aa, synthetic construct
QVQLVQSGSELKKPGESVKVSCKASGYTFTDYLVHWVRQAPGQGLEWMGWINTYTGTPTYADDFEGRFVFSLDTSVSTANLQISSLKAEDTAVYFCARSWRRGLRGIGFDYWGQGTLVTVSSASTKGPSVFPLAPSSKSTSGGTAALGCLVKDYFPEPVTVSWNSGALTSGVHTFPAVLQSSGLYSLSSVVTVPSSSLGTQTYICNVNHKPSNTKVDKRVEPKSCDKTHTCPPCPAPELLGGPSVFLFPPKPKDTLMISRTPEVTCVVVDVSHEDPEVKFNWYVDGVEVHNAKTKPREEQYNSTYRVVSVLTVLHQDWLNGKEYKCKVSNKALPAPIEKTISKAKGQPREPQVYTLPPSREEMTKNQVSLTCLVKGFYPSDIAVEWESNGQPENNYKTTPPVLDSDGSFFLYSKLTVDKSRWQQGNVFSCSVMHEALHNHYTQKSLSLSPGK

SEQ ID NO: 23 - protein, 452 aa, synthetic construct
QVQLVQSGPELKKPGESVKVSCKASGYTFTDYLVHWVRQAPGKGLEWMGWINTYTGTPTYADDFEGRFVFSLDTSASTANLQICSLKNEDTATYYCARSWRRGLRGIGFDYWGQGTLVTVSSASTKGPSVFPLAPSSKSTSGGTAALGCLVKDYFPEPVTVSWNSGALTSGVHTFPAVLQSSGLYSLSSVVTVPSSSLGTQTYICNVNHKPSNTKVDKRVEPKSCDKTHTCPPCPAPELLGGPSVFLFPPKPKDTLMISRTPEVTCVVVDVSHEDPEVKFNWYVDGVEVHNAKTKPREEQYNSTYRVVSVLTVLHQDWLNGKEYKCKVSNKALPAPIEKTISKAKGQPREPQVYTLPPSREEMTKNQVSLTCLVKGFYPSDIAVEWESNGQPENNYKTTPPVLDSDGSFFLYSKLTVDKSRWQQGNVFSCSVMHEALHNHYTQKSLSLSPGK

SEQ ID NO: 24 - protein, 214 aa, synthetic construct
DVQMTQSPYNLAASPGESVSINCKASKSINKYLAWYQQKPGKPNKLLIYDGSTLQSGIPSRFSGSGSGTDFTLTIRGLEPEDFGLYYCQQHNEYPPTFGAGTKLELKRTVAAPSVFIFPPSDEQLKSGTASVVCLLNNFYPREAKVQWKVDNALQSGNSQESVTEQDSKDSTYSLSSTLTLSKADYEKHKVYACEVTHQGLSSPVTKSFNRGEC

SEQ ID NO: 25 - protein, 214 aa, synthetic construct
DIQMTQSPYSLSASVGDRVTITCKASKSINKYLAWFQQKPGKPNKLLIYDGSTLQSGVPSRFSGSGSGTDFTLTISSLEPEDFATYYCQQHNEYPPTFGQGTKLEIKRTVAAPSVFIFPPSDEQLKSGTASVVCLLNNFYPREAKVQWKVDNALQSGNSQESVTEQDSKDSTYSLSSTLTLSKADYEKHKVYACEVTHQGLSSPVTKSFNRGEC